European Patent Specification EP 3 665 481 B1, published October 11, 2023. Title: Carbohydrate Sensors. Applicant: Commonwealth Scientific and Industrial Research Organisation. The sequence listing filed with the application follows.

SEQUENCE LISTING (74 sequences)

SEQ ID NO: 1 - protein, 279 aa, Artificial Sequence
  BgaR
MQILWKKYVKENFEMNVDECGIEQGIPGLGYNYEVLKNAVIHYVTKGYGTFKFNGKVYNLKQGDIFILLKGMQVEYVASIDDPWEYYWIGFSGSNANEYLNRTSITNSCVANCEENSKIPQIILNMCEISKTYNPSRSDDILLLKELYSLLYALIEEFPKPFEYKDKELHTYIQDALNFINSNYMHSITVQEIADYVNLSRSYLYKMFIKNLGISPQRYLINLRMYKATLLLKSTKLPIGEVASSVGYSDSLLFSKTFSKHFSMSPLNYRNNQVNKPSI

SEQ ID NO: 2 - protein, 6 aa, Artificial Sequence
  Linker sequence
GSSGGS

SEQ ID NO: 3 - protein, 6 aa, Artificial Sequence
  Linker sequence
GGSGGS

SEQ ID NO: 4 - protein, 6 aa, Artificial Sequence
  Linker sequence
GGTGGG

SEQ ID NO: 5 - protein, 6 aa, Artificial Sequence
  Linker sequence
GGGGGT

SEQ ID NO: 6 - protein, 8 aa, Artificial Sequence
  Linker sequence
LQGGTGGG

SEQ ID NO: 7 - protein, 8 aa, Artificial Sequence
  Linker sequence
FEGGTGGG

SEQ ID NO: 8 - protein, 7 aa, Artificial Sequence
  Linker sequence
GGSGGSL

SEQ ID NO: 9 - protein, 157 aa, Artificial Sequence
  BgaR putative CBD
MQILWKKYVKENFEMNVDECGIEQGIPGLGYNYEVLKNAVIHYVTKGYGTFKFNGKVYNLKQGDIFILLKGMQVEYVASIDDPWEYYWIGFSGSNANEYLNRTSITNSCVANCEENSKIPQIILNMCEISKTYNPSRSDDILLLKELYSLLYALIEE

SEQ ID NO: 10 - DNA, 26 bp, Artificial Sequence
  primer
aaaaaactgcagatgcagattctgtg

SEQ ID NO: 11 - DNA, 26 bp, Artificial Sequence
  primer
acacacttcgaaaatgctcggtttat

SEQ ID NO: 12 - DNA, 50 bp, Artificial Sequence
  primer
aaaaaactgcagggtggtaccggaggcggcatgcagattctgtggaaaaa

SEQ ID NO: 13 - DNA, 50 bp, Artificial Sequence
  primer
aaaaaattcgaagccgcctccggtaccaccaatgctcggtttattaactt

SEQ ID NO: 14 - DNA, 26 bp, Artificial Sequence
  Primer
aaaaaactgcagaatgctcggtttat

SEQ ID NO: 15 - protein, 833 aa, Artificial Sequence
  LacB1
MVSKGEELFTGVVPILVELDGDVNGHKFSVSGEGEGDATYGKLTLKFICTTGKLPVPWPTLVTTLSYGVQCFSRYPDHMKQHDFFKSAMPEGYVQERTIFFKDDGNYKTRAEVKFEGDTLVNRIELKGIDFKEDGNILGHKLEYNYNSHNVYIMADKQKNGIKVNFKIRHNIEDGSVQLADHYQQNTPIGDGPVLLPDNHYLSTQSALSKDPNEKRDHMVLLEFVTAAGITLGMDELYKLQMQILWKKYVKENFEMNVDECGIEQGIPGLGYNYEVLKNAVIHYVTKGYGTFKFNGKVYNLKQGDIFILLKGMQVEYVASIDDPWEYYWIGFSGSNANEYLNRTSITNSCVANCEENSKIPQIILNMCEISKTYNPSRSDDILLLKELYSLLYALIEEFPKPFEYKDKELHTYIQDALNFINSNYMHSITVQEIADYVNLSRSYLYKMFIKNLGISPQRYLINLRMYKATLLLKSTKLPIGEVASSVGYSDSLLFSKTFSKHFSMSPLNYRNNQVNKPSIFEMASKVYDPEQRKRMITGPQWWARCKQMNVLDSFINYYDSEKHAENAVIFLHGNATSSYLWRHVVPHIEPVARCIIPDLIGMGKSGKSGNGSYRLLDHYKYLTAWFELLNLPKKIIFVGHDWGAALAFHYAYEHQDRIKAIVHMESVVDVIESWDEWPDIEEDIALIKSEEGEKMVLENNFFVETVLPSKIMRKLEPEEFAAYLEPFKEKGEVRRPTLSWPREIPLVKGGKPDVVQIVRNYNAYLRASDDLPKLFIESDPGFFSNAIVEGAKKFPNTEFVKVKGLHFLQEDAPDEMGKYIKSFVERVLKNEQ

SEQ ID NO: 16 - protein, 845 aa, Artificial Sequence
  LacB2
MVSKGEELFTGVVPILVELDGDVNGHKFSVSGEGEGDATYGKLTLKFICTTGKLPVPWPTLVTTLSYGVQCFSRYPDHMKQHDFFKSAMPEGYVQERTIFFKDDGNYKTRAEVKFEGDTLVNRIELKGIDFKEDGNILGHKLEYNYNSHNVYIMADKQKNGIKVNFKIRHNIEDGSVQLADHYQQNTPIGDGPVLLPDNHYLSTQSALSKDPNEKRDHMVLLEFVTAAGITLGMDELYKLQGGTGGGMQILWKKYVKENFEMNVDECGIEQGIPGLGYNYEVLKNAVIHYVTKGYGTFKFNGKVYNLKQGDIFILLKGMQVEYVASIDDPWEYYWIGFSGSNANEYLNRTSITNSCVANCEENSKIPQIILNMCEISKTYNPSRSDDILLLKELYSLLYALIEEFPKPFEYKDKELHTYIQDALNFINSNYMHSITVQEIADYVNLSRSYLYKMFIKNLGISPQRYLINLRMYKATLLLKSTKLPIGEVASSVGYSDSLLFSKTFSKHFSMSPLNYRNNQVNKPSIFEGGTGGGMASKVYDPEQRKRMITGPQWWARCKQMNVLDSFINYYDSEKHAENAVIFLHGNATSSYLWRHVVPHIEPVARCIIPDLIGMGKSGKSGNGSYRLLDHYKYLTAWFELLNLPKKIIFVGHDWGAALAFHYAYEHQDRIKAIVHMESVVDVIESWDEWPDIEEDIALIKSEEGEKMVLENNFFVETVLPSKIMRKLEPEEFAAYLEPFKEKGEVRRPTLSWPREIPLVKGGKPDVVQIVRNYNAYLRASDDLPKLFIESDPGFFSNAIVEGAKKFPNTEFVKVKGLHFLQEDAPDEMGKYIKSFVERVLKNEQ

SEQ ID NO: 17 - protein, 839 aa, Artificial Sequence
  LacB3
MVSKGEELFTGVVPILVELDGDVNGHKFSVSGEGEGDATYGKLTLKFICTTGKLPVPWPTLVTTLSYGVQCFSRYPDHMKQHDFFKSAMPEGYVQERTIFFKDDGNYKTRAEVKFEGDTLVNRIELKGIDFKEDGNILGHKLEYNYNSHNVYIMADKQKNGIKVNFKIRHNIEDGSVQLADHYQQNTPIGDGPVLLPDNHYLSTQSALSKDPNEKRDHMVLLEFVTAAGITLGMDELYKLQGGTGGGMQILWKKYVKENFEMNVDECGIEQGIPGLGYNYEVLKNAVIHYVTKGYGTFKFNGKVYNLKQGDIFILLKGMQVEYVASIDDPWEYYWIGFSGSNANEYLNRTSITNSCVANCEENSKIPQIILNMCEISKTYNPSRSDDILLLKELYSLLYALIEEFPKPFEYKDKELHTYIQDALNFINSNYMHSITVQEIADYVNLSRSYLYKMFIKNLGISPQRYLINLRMYKATLLLKSTKLPIGEVASSVGYSDSLLFSKTFSKHFSMSPLNYRNNQVNKPSIFEMASKVYDPEQRKRMITGPQWWARCKQMNVLDSFINYYDSEKHAENAVIFLHGNATSSYLWRHVVPHIEPVARCIIPDLIGMGKSGKSGNGSYRLLDHYKYLTAWFELLNLPKKIIFVGHDWGAALAFHYAYEHQDRIKAIVHMESVVDVIESWDEWPDIEEDIALIKSEEGEKMVLENNFFVETVLPSKIMRKLEPEEFAAYLEPFKEKGEVRRPTLSWPREIPLVKGGKPDVVQIVRNYNAYLRASDDLPKLFIESDPGFFSNAIVEGAKKFPNTEFVKVKGLHFLQEDAPDEMGKYIKSFVERVLKNEQ

SEQ ID NO: 18 - protein, 839 aa, Artificial Sequence
  LacB4
MVSKGEELFTGVVPILVELDGDVNGHKFSVSGEGEGDATYGKLTLKFICTTGKLPVPWPTLVTTLSYGVQCFSRYPDHMKQHDFFKSAMPEGYVQERTIFFKDDGNYKTRAEVKFEGDTLVNRIELKGIDFKEDGNILGHKLEYNYNSHNVYIMADKQKNGIKVNFKIRHNIEDGSVQLADHYQQNTPIGDGPVLLPDNHYLSTQSALSKDPNEKRDHMVLLEFVTAAGITLGMDELYKLQMQILWKKYVKENFEMNVDECGIEQGIPGLGYNYEVLKNAVIHYVTKGYGTFKFNGKVYNLKQGDIFILLKGMQVEYVASIDDPWEYYWIGFSGSNANEYLNRTSITNSCVANCEENSKIPQIILNMCEISKTYNPSRSDDILLLKELYSLLYALIEEFPKPFEYKDKELHTYIQDALNFINSNYMHSITVQEIADYVNLSRSYLYKMFIKNLGISPQRYLINLRMYKATLLLKSTKLPIGEVASSVGYSDSLLFSKTFSKHFSMSPLNYRNNQVNKPSIFEGGTGGGMASKVYDPEQRKRMITGPQWWARCKQMNVLDSFINYYDSEKHAENAVIFLHGNATSSYLWRHVVPHIEPVARCIIPDLIGMGKSGKSGNGSYRLLDHYKYLTAWFELLNLPKKIIFVGHDWGAALAFHYAYEHQDRIKAIVHMESVVDVIESWDEWPDIEEDIALIKSEEGEKMVLENNFFVETVLPSKIMRKLEPEEFAAYLEPFKEKGEVRRPTLSWPREIPLVKGGKPDVVQIVRNYNAYLRASDDLPKLFIESDPGFFSNAIVEGAKKFPNTEFVKVKGLHFLQEDAPDEMGKYIKSFVERVLKNEQ

SEQ ID NO: 19 - DNA, 2502 bp, Artificial Sequence
  Nucleotide sequence encoding LacB1
atggtgagcaagggcgaggagctgttcaccggggtggtgcccatcctggtcgagctggacggcgacgtaaacggccacaagttcagcgtgtccggcgagggcgagggcgatgccacctacggcaagctgaccctgaagttcatctgcaccaccggcaagctgcccgtgccctggcccaccctcgtgaccaccctgagctacggcgtgcagtgcttcagccgctaccccgaccacatgaagcagcacgacttcttcaagtccgccatgcccgaaggctacgtccaggagcgcaccatcttcttcaaggacgacggcaactacaagacccgcgccgaggtgaagttcgagggcgacaccctggtgaaccgcatcgagctgaagggcatcgacttcaaggaggacggcaacatcctggggcacaagctggagtacaactacaacagccacaacgtctatatcatggccgacaagcagaagaacggcatcaaggtgaacttcaagatccgccacaacatcgaggacggcagcgtgcagctcgccgaccactaccagcagaacacccccatcggcgacggccccgtgctgctgcccgacaaccactacctgagcacccagtccgccctgagcaaagaccccaacgagaagcgcgatcacatggtcctgctggagttcgtgaccgccgccgggatcactctcggcatggacgagctgtacaagctgcagatgcagattctgtggaaaaaatacgtcaaagaaaactttgaaatgaacgtggatgaatgcggcattgaacaaggcattccgggcctgggttataactacgaagttctgaaaaatgcagtcatccattatgtgaccaaaggctatggtacgtttaaattcaacggcaaagtctataatctgaaacagggtgacattttcatcctgctgaaaggcatgcaagtggaatacgttgcgagcattgatgacccgtgggaatattactggatcggctttagtggttccaacgcgaatgaatatctgaaccgtaccagcattaccaacagctgcgtggccaactgtgaagaaaatagcaaaattccgcagattatcctgaacatgtgtgaaatctctaaaacctacaacccgtcacgctcggatgacattctgctgctgaaagaactgtattccctgctgtacgcactgatcgaagaatttccgaaaccgtttgaatacaaagataaagaactgcatacctacattcaggacgcgctgaacttcatcaactcaaattatatgcactcgattacggtgcaagaaatcgccgattacgttaatctgagccgttcttacctgtacaaaatgttcatcaaaaacctgggtatcagtccgcagcgttatctgattaatctgcgcatgtacaaagcaaccctgctgctgaaatctacgaaactgccgatcggcgaagttgcgagcagcgtgggttatagtgattccctgctgtttagtaaaaccttctccaaacacttttcaatgtcgccgctgaactaccgcaacaatcaagttaataaaccgagcattttcgaaatggcttccaaggtgtacgaccccgagcaacgcaaacgcatgatcactgggcctcagtggtgggctcgctgcaagcaaatgaacgtgctggactccttcatcaactactatgattccgagaagcacgccgagaacgccgtgatttttctgcatggtaacgctacctccagctacctgtggaggcacgtcgtgcctcacatcgagcccgtggctagatgcatcatccctgatctgatcggaatgggtaagtccggcaagagcgggaatggctcatatcgcctcctggatcactacaagtacctcaccgcttggttcgagctgctgaaccttccaaagaaaatcatctttgtgggccacgactggggggctgctctggcctttcactacgcctacgagcaccaagacaggatcaaggccatcgtccatatggagagtgtcgtggacgtgatcgagtcctgggacgagtggcctgacatcgaggaggatatcgccctgatcaagagcgaagagggcgagaaaatggtgcttgagaataacttcttcgtcgagaccgtgctcccaagcaagatcatgcggaaactggagcctgaggagttcgctgcctacctggagccattcaaggagaagggcgaggttagacggcctaccctctcctggcctcgcgagatccctctcgttaagggaggcaagcccgacgtcgtccagattgtccgcaactacaacgcctaccttcgggccagcgacgatctgcctaagctgttcatcgagtccgaccctgggttcttttccaacgctattgtcgagggagctaagaagttccctaacaccgagttcgtgaaggtgaagggcctccacttcctccaggaggacgctccagatgaaatgggtaagtacatcaagagcttcgtggagcgcgtgctgaagaacgagcagtaa

SEQ ID NO: 20 - DNA, 2538 bp, Artificial Sequence
  Nucleotide sequence encoding LacB2
atggtgagcaagggcgaggagctgttcaccggggtggtgcccatcctggtcgagctggacggcgacgtaaacggccacaagttcagcgtgtccggcgagggcgagggcgatgccacctacggcaagctgaccctgaagttcatctgcaccaccggcaagctgcccgtgccctggcccaccctcgtgaccaccctgagctacggcgtgcagtgcttcagccgctaccccgaccacatgaagcagcacgacttcttcaagtccgccatgcccgaaggctacgtccaggagcgcaccatcttcttcaaggacgacggcaactacaagacccgcgccgaggtgaagttcgagggcgacaccctggtgaaccgcatcgagctgaagggcatcgacttcaaggaggacggcaacatcctggggcacaagctggagtacaactacaacagccacaacgtctatatcatggccgacaagcagaagaacggcatcaaggtgaacttcaagatccgccacaacatcgaggacggcagcgtgcagctcgccgaccactaccagcagaacacccccatcggcgacggccccgtgctgctgcccgacaaccactacctgagcacccagtccgccctgagcaaagaccccaacgagaagcgcgatcacatggtcctgctggagttcgtgaccgccgccgggatcactctcggcatggacgagctgtacaagctgcagggtggtaccggaggcggcatgcagattctgtggaaaaaatacgtcaaagaaaactttgaaatgaacgtggatgaatgcggcattgaacaaggcattccgggcctgggttataactacgaagttctgaaaaatgcagtcatccattatgtgaccaaaggctatggtacgtttaaattcaacggcaaagtctataatctgaaacagggtgacattttcatcctgctgaaaggcatgcaagtggaatacgttgcgagcattgatgacccgtgggaatattactggatcggctttagtggttccaacgcgaatgaatatctgaaccgtaccagcattaccaacagctgcgtggccaactgtgaagaaaatagcaaaattccgcagattatcctgaacatgtgtgaaatctctaaaacctacaacccgtcacgctcggatgacattctgctgctgaaagaactgtattccctgctgtacgcactgatcgaagaatttccgaaaccgtttgaatacaaagataaagaactgcatacctacattcaggacgcgctgaacttcatcaactcaaattatatgcactcgattacggtgcaagaaatcgccgattacgttaatctgagccgttcttacctgtacaaaatgttcatcaaaaacctgggtatcagtccgcagcgttatctgattaatctgcgcatgtacaaagcaaccctgctgctgaaatctacgaaactgccgatcggcgaagttgcgagcagcgtgggttatagtgattccctgctgtttagtaaaaccttctccaaacacttttcaatgtcgccgctgaactaccgcaacaatcaagttaataaaccgagcattttcgaaggtggtaccggaggcggcatggcttccaaggtgtacgaccccgagcaacgcaaacgcatgatcactgggcctcagtggtgggctcgctgcaagcaaatgaacgtgctggactccttcatcaactactatgattccgagaagcacgccgagaacgccgtgatttttctgcatggtaacgctacctccagctacctgtggaggcacgtcgtgcctcacatcgagcccgtggctagatgcatcatccctgatctgatcggaatgggtaagtccggcaagagcgggaatggctcatatcgcctcctggatcactacaagtacctcaccgcttggttcgagctgctgaaccttccaaagaaaatcatctttgtgggccacgactggggggctgctctggcctttcactacgcctacgagcaccaagacaggatcaaggccatcgtccatatggagagtgtcgtggacgtgatcgagtcctgggacgagtggcctgacatcgaggaggatatcgccctgatcaagagcgaagagggcgagaaaatggtgcttgagaataacttcttcgtcgagaccgtgctcccaagcaagatcatgcggaaactggagcctgaggagttcgctgcctacctggagccattcaaggagaagggcgaggttagacggcctaccctctcctggcctcgcgagatccctctcgttaagggaggcaagcccgacgtcgtccagattgtccgcaactacaacgcctaccttcgggccagcgacgatctgcctaagctgttcatcgagtccgaccctgggttcttttccaacgctattgtcgagggagctaagaagttccctaacaccgagttcgtgaaggtgaagggcctccacttcctccaggaggacgctccagatgaaatgggtaagtacatcaagagcttcgtggagcgcgtgctgaagaacgagcagtaa

SEQ ID NO: 21 - DNA, 2520 bp, Artificial Sequence
  Nucleotide sequence encoding LacB3
atggtgagcaagggcgaggagctgttcaccggggtggtgcccatcctggtcgagctggacggcgacgtaaacggccacaagttcagcgtgtccggcgagggcgagggcgatgccacctacggcaagctgaccctgaagttcatctgcaccaccggcaagctgcccgtgccctggcccaccctcgtgaccaccctgagctacggcgtgcagtgcttcagccgctaccccgaccacatgaagcagcacgacttcttcaagtccgccatgcccgaaggctacgtccaggagcgcaccatcttcttcaaggacgacggcaactacaagacccgcgccgaggtgaagttcgagggcgacaccctggtgaaccgcatcgagctgaagggcatcgacttcaaggaggacggcaacatcctggggcacaagctggagtacaactacaacagccacaacgtctatatcatggccgacaagcagaagaacggcatcaaggtgaacttcaagatccgccacaacatcgaggacggcagcgtgcagctcgccgaccactaccagcagaacacccccatcggcgacggccccgtgctgctgcccgacaaccactacctgagcacccagtccgccctgagcaaagaccccaacgagaagcgcgatcacatggtcctgctggagttcgtgaccgccgccgggatcactctcggcatggacgagctgtacaagctgcagggtggtaccggaggcggcatgcagattctgtggaaaaaatacgtcaaagaaaactttgaaatgaacgtggatgaatgcggcattgaacaaggcattccgggcctgggttataactacgaagttctgaaaaatgcagtcatccattatgtgaccaaaggctatggtacgtttaaattcaacggcaaagtctataatctgaaacagggtgacattttcatcctgctgaaaggcatgcaagtggaatacgttgcgagcattgatgacccgtgggaatattactggatcggctttagtggttccaacgcgaatgaatatctgaaccgtaccagcattaccaacagctgcgtggccaactgtgaagaaaatagcaaaattccgcagattatcctgaacatgtgtgaaatctctaaaacctacaacccgtcacgctcggatgacattctgctgctgaaagaactgtattccctgctgtacgcactgatcgaagaatttccgaaaccgtttgaatacaaagataaagaactgcatacctacattcaggacgcgctgaacttcatcaactcaaattatatgcactcgattacggtgcaagaaatcgccgattacgttaatctgagccgttcttacctgtacaaaatgttcatcaaaaacctgggtatcagtccgcagcgttatctgattaatctgcgcatgtacaaagcaaccctgctgctgaaatctacgaaactgccgatcggcgaagttgcgagcagcgtgggttatagtgattccctgctgtttagtaaaaccttctccaaacacttttcaatgtcgccgctgaactaccgcaacaatcaagttaataaaccgagcattttcgaaatggcttccaaggtgtacgaccccgagcaacgcaaacgcatgatcactgggcctcagtggtgggctcgctgcaagcaaatgaacgtgctggactccttcatcaactactatgattccgagaagcacgccgagaacgccgtgatttttctgcatggtaacgctacctccagctacctgtggaggcacgtcgtgcctcacatcgagcccgtggctagatgcatcatccctgatctgatcggaatgggtaagtccggcaagagcgggaatggctcatatcgcctcctggatcactacaagtacctcaccgcttggttcgagctgctgaaccttccaaagaaaatcatctttgtgggccacgactggggggctgctctggcctttcactacgcctacgagcaccaagacaggatcaaggccatcgtccatatggagagtgtcgtggacgtgatcgagtcctgggacgagtggcctgacatcgaggaggatatcgccctgatcaagagcgaagagggcgagaaaatggtgcttgagaataacttcttcgtcgagaccgtgctcccaagcaagatcatgcggaaactggagcctgaggagttcgctgcctacctggagccattcaaggagaagggcgaggttagacggcctaccctctcctggcctcgcgagatccctctcgttaagggaggcaagcccgacgtcgtccagattgtccgcaactacaacgcctaccttcgggccagcgacgatctgcctaagctgttcatcgagtccgaccctgggttcttttccaacgctattgtcgagggagctaagaagttccctaacaccgagttcgtgaaggtgaagggcctccacttcctccaggaggacgctccagatgaaatgggtaagtacatcaagagcttcgtggagcgcgtgctgaagaacgagcagtaa

SEQ ID NO: 22 - DNA, 2520 bp, Artificial Sequence
  Nucleotide sequence encoding LacB4
atggtgagcaagggcgaggagctgttcaccggggtggtgcccatcctggtcgagctggacggcgacgtaaacggccacaagttcagcgtgtccggcgagggcgagggcgatgccacctacggcaagctgaccctgaagttcatctgcaccaccggcaagctgcccgtgccctggcccaccctcgtgaccaccctgagctacggcgtgcagtgcttcagccgctaccccgaccacatgaagcagcacgacttcttcaagtccgccatgcccgaaggctacgtccaggagcgcaccatcttcttcaaggacgacggcaactacaagacccgcgccgaggtgaagttcgagggcgacaccctggtgaaccgcatcgagctgaagggcatcgacttcaaggaggacggcaacatcctggggcacaagctggagtacaactacaacagccacaacgtctatatcatggccgacaagcagaagaacggcatcaaggtgaacttcaagatccgccacaacatcgaggacggcagcgtgcagctcgccgaccactaccagcagaacacccccatcggcgacggccccgtgctgctgcccgacaaccactacctgagcacccagtccgccctgagcaaagaccccaacgagaagcgcgatcacatggtcctgctggagttcgtgaccgccgccgggatcactctcggcatggacgagctgtacaagctgcagatgcagattctgtggaaaaaatacgtcaaagaaaactttgaaatgaacgtggatgaatgcggcattgaacaaggcattccgggcctgggttataactacgaagttctgaaaaatgcagtcatccattatgtgaccaaaggctatggtacgtttaaattcaacggcaaagtctataatctgaaacagggtgacattttcatcctgctgaaaggcatgcaagtggaatacgttgcgagcattgatgacccgtgggaatattactggatcggctttagtggttccaacgcgaatgaatatctgaaccgtaccagcattaccaacagctgcgtggccaactgtgaagaaaatagcaaaattccgcagattatcctgaacatgtgtgaaatctctaaaacctacaacccgtcacgctcggatgacattctgctgctgaaagaactgtattccctgctgtacgcactgatcgaagaatttccgaaaccgtttgaatacaaagataaagaactgcatacctacattcaggacgcgctgaacttcatcaactcaaattatatgcactcgattacggtgcaagaaatcgccgattacgttaatctgagccgttcttacctgtacaaaatgttcatcaaaaacctgggtatcagtccgcagcgttatctgattaatctgcgcatgtacaaagcaaccctgctgctgaaatctacgaaactgccgatcggcgaagttgcgagcagcgtgggttatagtgattccctgctgtttagtaaaaccttctccaaacacttttcaatgtcgccgctgaactaccgcaacaatcaagttaataaaccgagcattttcgaaggtggtaccggaggcggcatggcttccaaggtgtacgaccccgagcaacgcaaacgcatgatcactgggcctcagtggtgggctcgctgcaagcaaatgaacgtgctggactccttcatcaactactatgattccgagaagcacgccgagaacgccgtgatttttctgcatggtaacgctacctccagctacctgtggaggcacgtcgtgcctcacatcgagcccgtggctagatgcatcatccctgatctgatcggaatgggtaagtccggcaagagcgggaatggctcatatcgcctcctggatcactacaagtacctcaccgcttggttcgagctgctgaaccttccaaagaaaatcatctttgtgggccacgactggggggctgctctggcctttcactacgcctacgagcaccaagacaggatcaaggccatcgtccatatggagagtgtcgtggacgtgatcgagtcctgggacgagtggcctgacatcgaggaggatatcgccctgatcaagagcgaagagggcgagaaaatggtgcttgagaataacttcttcgtcgagaccgtgctcccaagcaagatcatgcggaaactggagcctgaggagttcgctgcctacctggagccattcaaggagaagggcgaggttagacggcctaccctctcctggcctcgcgagatccctctcgttaagggaggcaagcccgacgtcgtccagattgtccgcaactacaacgcctaccttcgggccagcgacgatctgcctaagctgttcatcgagtccgaccctgggttcttttccaacgctattgtcgagggagctaagaagttccctaacaccgagttcgtgaaggtgaagggcctccacttcctccaggaggacgctccagatgaaatgggtaagtacatcaagagcttcgtggagcgcgtgctgaagaacgagcagtaa

SEQ ID NO: 23 - protein, 799 aa, Artificial Sequence
  LacF1
MRGSHHHHHHGMASMTGGQQMGRDLYDDDDKDRWGSEFMVSKGEELFTGVVPILVELDGDVNGHRFSVSGEGEGDATYGKLTLKFICTTGKLPVPWPTLVTTLTWGVQCFSRYPDHMKQHDFFKSAMPEGYVQERTIFFKDDGNYKTRAEVKFEGDTLVNRIELKGIDFKEDGNILGHKLEYNYISHNVYITADKQKNGIKAHFKIRHNIEDGSVQLADHYQQNTPIGDGPVLLPDNHYLSTQSALSKDPNEKRDHMVLLEFVTAAGITLGMDELYKLQMQILWKKYVKENFEMNVDECGIEQGIPGLGYNYEVLKNAVIHYVTKGYGTFKFNGKVYNLKQGDIFILLKGMQVEYVASIDDPWEYYWIGFSGSNANEYLNRTSITNSCVANCEENSKIPQIILNMCEISKTYNPSRSDDILLLKELYSLLYALIEEFPKPFEYKDKELHTYIQDALNFINSNYMHSITVQEIADYVNLSRSYLYKMFIKNLGISPQRYLINLRMYKATLLLKSTKLPIGEVASSVGYSDSLLFSKTFSKHFSMSPLNYRNNQVNKPSIFEMVSKGEELFTGVVPILVELDGDVNGHKFSVSGEGEGDATYGKLTLKFICTTGKLPVPWPTLVTTFGYGVQCFARYPDHMRQHDFFKSAMPEGYVQERTIFFKDDGNYKTRAEVKFEGDTLVNRIELKGIDFKEDGNILGHKLEYNYNSHNVYIMADKQKNGIKVNFKIRHNIEDGSVQLADHYQQNTPIGDGPVLLPDNHYLSYQSALSKDPNEKRDHMVLLEFVTAAGITLGMDELYK

SEQ ID NO: 24 - DNA, 2397 bp, Artificial Sequence
  Nucleotide sequence encoding LacF1
atgcggggttctcatcatcatcatcatcatggtatggctagcatgactggtggacagcaaatgggtcgggatctgtacgacgatgacgataaggatcgatggggatccgaattcatggtgagcaagggcgaggagctgttcaccggggtggtgcccatcctggtcgagctggacggcgacgtaaacggccacaggttcagcgtgtccggcgagggcgagggcgatgccacctacggcaagctgaccctgaagttcatctgcaccaccggcaagctgcccgtgccctggcccaccctcgtgaccaccctgacctggggcgtgcagtgcttcagccgctaccccgaccacatgaagcagcacgacttcttcaagtccgccatgcccgaaggctacgtccaggagcgtaccatcttcttcaaggacgacggcaactacaagacccgcgccgaggtgaagttcgagggcgacaccctggtgaaccgcatcgagctgaagggcatcgacttcaaggaggacggcaacatcctggggcacaagctggagtacaactacatcagccacaacgtctatatcaccgccgacaagcagaagaacggcatcaaggcccacttcaagatccgccacaacatcgaggacggcagcgtgcagctcgccgaccactaccagcagaacacccccatcggcgacggccccgtgctgctgcccgacaaccactacctgagcacccagtccgccctgagcaaagaccccaacgagaagcgcgatcacatggtcctgctggagttcgtgaccgccgccgggatcactctcggcatggacgagctgtacaagctgcagatgcagattctgtggaaaaaatacgtcaaagaaaactttgaaatgaacgtggatgaatgcggcattgaacaaggcattccgggcctgggttataactacgaagttctgaaaaatgcagtcatccattatgtgaccaaaggctatggtacgtttaaattcaacggcaaagtctataatctgaaacagggtgacattttcatcctgctgaaaggcatgcaagtggaatacgttgcgagcattgatgacccgtgggaatattactggatcggctttagtggttccaacgcgaatgaatatctgaaccgtaccagcattaccaacagctgcgtggccaactgtgaagaaaatagcaaaattccgcagattatcctgaacatgtgtgaaatctctaaaacctacaacccgtcacgctcggatgacattctgctgctgaaagaactgtattccctgctgtacgcactgatcgaagaatttccgaaaccgtttgaatacaaagataaagaactgcatacctacattcaggacgcgctgaacttcatcaactcaaattatatgcactcgattacggtgcaagaaatcgccgattacgttaatctgagccgttcttacctgtacaaaatgttcatcaaaaacctgggtatcagtccgcagcgttatctgattaatctgcgcatgtacaaagcaaccctgctgctgaaatctacgaaactgccgatcggcgaagttgcgagcagcgtgggttatagtgattccctgctgtttagtaaaaccttctccaaacacttttcaatgtcgccgctgaactaccgcaacaatcaagttaataaaccgagcattctgcagatggtgagcaagggcgaggagctgttcaccggggtggtgcccatcctggtcgagctggacggcgacgtaaacggccacaagttcagcgtgtccggcgagggcgagggcgatgccacctacggcaagctgaccctgaagttcatctgcaccaccggcaagctgcccgtgccctggcccaccctcgtgaccaccttcggctacggcgtgcagtgcttcgcccgctaccccgaccacatgcgccagcacgacttcttcaagtccgccatgcccgaaggctacgtccaggagcgcaccatcttcttcaaggacgacggcaactacaagacccgcgccgaggtgaagttcgagggcgacaccctggtgaaccgcatcgagctgaagggcatcgacttcaaggaggacggcaacatcctggggcacaagctggagtacaactacaacagccacaacgtctatatcatggccgacaagcagaagaacggcatcaaggtgaacttcaagatccgccacaacatcgaggacggcagcgtgcagctcgccgaccactaccagcagaacacccccatcggcgacggccccgtgctgctgcccgacaaccactacctgagctaccagtccgccctgagcaaagaccccaacgagaagcgcgatcacatggtcctgctggagttcgtgaccgccgccgggatcactctcggcatggacgagctgtacaag

SEQ ID NO: 25 - protein, 873 aa, Artificial Sequence
  LacB1
MRGSHHHHHHGMASMTGGQQMGRDLYDDDDKDRWGSEFMVSKGEELFTGVVPILVELDGDVNGHKFSVSGEGEGDATYGKLTLKFICTTGKLPVPWPTLVTTLSYGVQCFSRYPDHMKQHDFFKSAMPEGYVQERTIFFKDDGNYKTRAEVKFEGDTLVNRIELKGIDFKEDGNILGHKLEYNYNSHNVYIMADKQKNGIKVNFKIRHNIEDGSVQLADHYQQNTPIGDGPVLLPDNHYLSTQSALSKDPNEKRDHMVLLEFVTAAGITLGMDELYKLQMQILWKKYVKENFEMNVDECGIEQGIPGLGYNYEVLKNAVIHYVTKGYGTFKFNGKVYNLKQGDIFILLKGMQVEYVASIDDPWEYYWIGFSGSNANEYLNRTSITNSCVANCEENSKIPQIILNMCEISKTYNPSRSDDILLLKELYSLLYALIEEFPKPFEYKDKELHTYIQDALNFINSNYMHSITVQEIADYVNLSRSYLYKMFIKNLGISPQRYLINLRMYKATLLLKSTKLPIGEVASSVGYSDSLLFSKTFSKHFSMSPLNYRNNQVNKPSIFELQMASKVYDPEQRKRMITGPQWWARCKQMNVLDSFINYYDSEKHAENAVIFLHGNATSSYLWRHVVPHIEPVARCIIPDLIGMGKSGKSGNGSYRLLDHYKYLTAWFELLNLPKKIIFVGHDWGAALAFHYAYEHQDRIKAIVHMESVVDVIESWDEWPDIEEDIALIKSEEGEKMVLENNFFVETVLPSKIMRKLEPEEFAAYLEPFKEKGEVRRPTLSWPREIPLVKGGKPDVVQIVRNYNAYLRASDDLPKLFIESDPGFFSNAIVEGAKKFPNTEFVKVKGLHFLQEDAPDEMGKYIKSFVERVLKNEQ

SEQ ID NO: 26 - protein, 885 aa, Artificial Sequence
  LacB2
MRGSHHHHHHGMASMTGGQQMGRDLYDDDDKDRWGSEFMVSKGEELFTGVVPILVELDGDVNGHKFSVSGEGEGDATYGKLTLKFICTTGKLPVPWPTLVTTLSYGVQCFSRYPDHMKQHDFFKSAMPEGYVQERTIFFKDDGNYKTRAEVKFEGDTLVNRIELKGIDFKEDGNILGHKLEYNYNSHNVYIMADKQKNGIKVNFKIRHNIEDGSVQLADHYQQNTPIGDGPVLLPDNHYLSTQSALSKDPNEKRDHMVLLEFVTAAGITLGMDELYKLQGGTGGGMQILWKKYVKENFEMNVDECGIEQGIPGLGYNYEVLKNAVIHYVTKGYGTFKFNGKVYNLKQGDIFILLKGMQVEYVASIDDPWEYYWIGFSGSNANEYLNRTSITNSCVANCEENSKIPQIILNMCEISKTYNPSRSDDILLLKELYSLLYALIEEFPKPFEYKDKELHTYIQDALNFINSNYMHSITVQEIADYVNLSRSYLYKMFIKNLGISPQRYLINLRMYKATLLLKSTKLPIGEVASSVGYSDSLLFSKTFSKHFSMSPLNYRNNQVNKPSIGGTGGGFELQMASKVYDPEQRKRMITGPQWWARCKQMNVLDSFINYYDSEKHAENAVIFLHGNATSSYLWRHVVPHIEPVARCIIPDLIGMGKSGKSGNGSYRLLDHYKYLTAWFELLNLPKKIIFVGHDWGAALAFHYAYEHQDRIKAIVHMESVVDVIESWDEWPDIEEDIALIKSEEGEKMVLENNFFVETVLPSKIMRKLEPEEFAAYLEPFKEKGEVRRPTLSWPREIPLVKGGKPDVVQIVRNYNAYLRASDDLPKLFIESDPGFFSNAIVEGAKKFPNTEFVKVKGLHFLQEDAPDEMGKYIKSFVERVLKNEQ

SEQ ID NO: 27 - protein, 879 aa, Artificial Sequence
  LacB3
MRGSHHHHHHGMASMTGGQQMGRDLYDDDDKDRWGSEFMVSKGEELFTGVVPILVELDGDVNGHKFSVSGEGEGDATYGKLTLKFICTTGKLPVPWPTLVTTLSYGVQCFSRYPDHMKQHDFFKSAMPEGYVQERTIFFKDDGNYKTRAEVKFEGDTLVNRIELKGIDFKEDGNILGHKLEYNYNSHNVYIMADKQKNGIKVNFKIRHNIEDGSVQLADHYQQNTPIGDGPVLLPDNHYLSTQSALSKDPNEKRDHMVLLEFVTAAGITLGMDELYKLQGGTGGGMQILWKKYVKENFEMNVDECGIEQGIPGLGYNYEVLKNAVIHYVTKGYGTFKFNGKVYNLKQGDIFILLKGMQVEYVASIDDPWEYYWIGFSGSNANEYLNRTSITNSCVANCEENSKIPQIILNMCEISKTYNPSRSDDILLLKELYSLLYALIEEFPKPFEYKDKELHTYIQDALNFINSNYMHSITVQEIADYVNLSRSYLYKMFIKNLGISPQRYLINLRMYKATLLLKSTKLPIGEVASSVGYSDSLLFSKTFSKHFSMSPLNYRNNQVNKPSIFELQMASKVYDPEQRKRMITGPQWWARCKQMNVLDSFINYYDSEKHAENAVIFLHGNATSSYLWRHVVPHIEPVARCIIPDLIGMGKSGKSGNGSYRLLDHYKYLTAWFELLNLPKKIIFVGHDWGAALAFHYAYEHQDRIKAIVHMESVVDVIESWDEWPDIEEDIALIKSEEGEKMVLENNFFVETVLPSKIMRKLEPEEFAAYLEPFKEKGEVRRPTLSWPREIPLVKGGKPDVVQIVRNYNAYLRASDDLPKLFIESDPGFFSNAIVEGAKKFPNTEFVKVKGLHFLQEDAPDEMGKYIKSFVERVLKNEQ

SEQ ID NO: 28 - protein, 879 aa, Artificial Sequence
  LacB4
MRGSHHHHHHGMASMTGGQQMGRDLYDDDDKDRWGSEFMVSKGEELFTGVVPILVELDGDVNGHKFSVSGEGEGDATYGKLTLKFICTTGKLPVPWPTLVTTLSYGVQCFSRYPDHMKQHDFFKSAMPEGYVQERTIFFKDDGNYKTRAEVKFEGDTLVNRIELKGIDFKEDGNILGHKLEYNYNSHNVYIMADKQKNGIKVNFKIRHNIEDGSVQLADHYQQNTPIGDGPVLLPDNHYLSTQSALSKDPNEKRDHMVLLEFVTAAGITLGMDELYKLQMQILWKKYVKENFEMNVDECGIEQGIPGLGYNYEVLKNAVIHYVTKGYGTFKFNGKVYNLKQGDIFILLKGMQVEYVASIDDPWEYYWIGFSGSNANEYLNRTSITNSCVANCEENSKIPQIILNMCEISKTYNPSRSDDILLLKELYSLLYALIEEFPKPFEYKDKELHTYIQDALNFINSNYMHSITVQEIADYVNLSRSYLYKMFIKNLGISPQRYLINLRMYKATLLLKSTKLPIGEVASSVGYSDSLLFSKTFSKHFSMSPLNYRNNQVNKPSIGGTGGGFELQMASKVYDPEQRKRMITGPQWWARCKQMNVLDSFINYYDSEKHAENAVIFLHGNATSSYLWRHVVPHIEPVARCIIPDLIGMGKSGKSGNGSYRLLDHYKYLTAWFELLNLPKKIIFVGHDWGAALAFHYAYEHQDRIKAIVHMESVVDVIESWDEWPDIEEDIALIKSEEGEKMVLENNFFVETVLPSKIMRKLEPEEFAAYLEPFKEKGEVRRPTLSWPREIPLVKGGKPDVVQIVRNYNAYLRASDDLPKLFIESDPGFFSNAIVEGAKKFPNTEFVKVKGLHFLQEDAPDEMGKYIKSFVERVLKNEQ

SEQ ID NO: 29 - DNA, 2622 bp, Artificial Sequence
  Nucleotide sequence encoding LacB1
atgcggggttctcatcatcatcatcatcatggtatggctagcatgactggtggacagcaaatgggtcgggatctgtacgacgatgacgataaggatcgatggggatccgaattcatggtgagcaagggcgaggagctgttcaccggggtggtgcccatcctggtcgagctggacggcgacgtaaacggccacaagttcagcgtgtccggcgagggcgagggcgatgccacctacggcaagctgaccctgaagttcatctgcaccaccggcaagctgcccgtgccctggcccaccctcgtgaccaccctgagctacggcgtgcagtgcttcagccgctaccccgaccacatgaagcagcacgacttcttcaagtccgccatgcccgaaggctacgtccaggagcgcaccatcttcttcaaggacgacggcaactacaagacccgcgccgaggtgaagttcgagggcgacaccctggtgaaccgcatcgagctgaagggcatcgacttcaaggaggacggcaacatcctggggcacaagctggagtacaactacaacagccacaacgtctatatcatggccgacaagcagaagaacggcatcaaggtgaacttcaagatccgccacaacatcgaggacggcagcgtgcagctcgccgaccactaccagcagaacacccccatcggcgacggccccgtgctgctgcccgacaaccactacctgagcacccagtccgccctgagcaaagaccccaacgagaagcgcgatcacatggtcctgctggagttcgtgaccgccgccgggatcactctcggcatggacgagctgtacaagctgcagatgcagattctgtggaaaaaatacgtcaaagaaaactttgaaatgaacgtggatgaatgcggcattgaacaaggcattccgggcctgggttataactacgaagttctgaaaaatgcagtcatccattatgtgaccaaaggctatggtacgtttaaattcaacggcaaagtctataatctgaaacagggtgacattttcatcctgctgaaaggcatgcaagtggaatacgttgcgagcattgatgacccgtgggaatattactggatcggctttagtggttccaacgcgaatgaatatctgaaccgtaccagcattaccaacagctgcgtggccaactgtgaagaaaatagcaaaattccgcagattatcctgaacatgtgtgaaatctctaaaacctacaacccgtcacgctcggatgacattctgctgctgaaagaactgtattccctgctgtacgcactgatcgaagaatttccgaaaccgtttgaatacaaagataaagaactgcatacctacattcaggacgcgctgaacttcatcaactcaaattatatgcactcgattacggtgcaagaaatcgccgattacgttaatctgagccgttcttacctgtacaaaatgttcatcaaaaacctgggtatcagtccgcagcgttatctgattaatctgcgcatgtacaaagcaaccctgctgctgaaatctacgaaactgccgatcggcgaagttgcgagcagcgtgggttatagtgattccctgctgtttagtaaaaccttctccaaacacttttcaatgtcgccgctgaactaccgcaacaatcaagttaataaaccgagcattttcgaacttcagatggcttccaaggtgtacgaccccgagcaacgcaaacgcatgatcactgggcctcagtggtgggctcgctgcaagcaaatgaacgtgctggactccttcatcaactactatgattccgagaagcacgccgagaacgccgtgatttttctgcatggtaacgctacctccagctacctgtggaggcacgtcgtgcctcacatcgagcccgtggctagatgcatcatccctgatctgatcggaatgggtaagtccggcaagagcgggaatggctcatatcgcctcctggatcactacaagtacctcaccgcttggttcgagctgctgaaccttccaaagaaaatcatctttgtgggccacgactggggggctgctctggcctttcactacgcctacgagcaccaagacaggatcaaggccatcgtccatatggagagtgtcgtggacgtgatcgagtcctgggacgagtggcctgacatcgaggaggatatcgccctgatcaagagcgaagagggcgagaaaatggtgcttgagaataacttcttcgtcgagaccgtgctcccaagcaagatcatgcggaaactggagcctgaggagttcgctgcctacctggagccattcaaggagaagggcgaggttagacggcctaccctctcctggcctcgcgagatccctctcgttaagggaggcaagcccgacgtcgtccagattgtccgcaactacaacgcctaccttcgggccagcgacgatctgcctaagctgttcatcgagtccgaccctgggttcttttccaacgctattgtcgagggagctaagaagttccctaacaccgagttcgtgaaggtgaagggcctccacttcctccaggaggacgctccagatgaaatgggtaagtacatcaagagcttcgtggagcgcgtgctgaagaacgagcagtaa

SEQ ID NO: 30 - DNA, 2658 bp, Artificial Sequence
  Nucleotide sequence encoding LacB2
atgcggggttctcatcatcatcatcatcatggtatggctagcatgactggtggacagcaaatgggtcgggatctgtacgacgatgacgataaggatcgatggggatccgaattcatggtgagcaagggcgaggagctgttcaccggggtggtgcccatcctggtcgagctggacggcgacgtaaacggccacaagttcagcgtgtccggcgagggcgagggcgatgccacctacggcaagctgaccctgaagttcatctgcaccaccggcaagctgcccgtgccctggcccaccctcgtgaccaccctgagctacggcgtgcagtgcttcagccgctaccccgaccacatgaagcagcacgacttcttcaagtccgccatgcccgaaggctacgtccaggagcgcaccatcttcttcaaggacgacggcaactacaagacccgcgccgaggtgaagttcgagggcgacaccctggtgaaccgcatcgagctgaagggcatcgacttcaaggaggacggcaacatcctggggcacaagctggagtacaactacaacagccacaacgtctatatcatggccgacaagcagaagaacggcatcaaggtgaacttcaagatccgccacaacatcgaggacggcagcgtgcagctcgccgaccactaccagcagaacacccccatcggcgacggccccgtgctgctgcccgacaaccactacctgagcacccagtccgccctgagcaaagaccccaacgagaagcgcgatcacatggtcctgctggagttcgtgaccgccgccgggatcactctcggcatggacgagctgtacaagctgcagggtggtaccggaggcggcatgcagattctgtggaaaaaatacgtcaaagaaaactttgaaatgaacgtggatgaatgcggcattgaacaaggcattccgggcctgggttataactacgaagttctgaaaaatgcagtcatccattatgtgaccaaaggctatggtacgtttaaattcaacggcaaagtctataatctgaaacagggtgacattttcatcctgctgaaaggcatgcaagtggaatacgttgcgagcattgatgacccgtgggaatattactggatcggctttagtggttccaacgcgaatgaatatctgaaccgtaccagcattaccaacagctgcgtggccaactgtgaagaaaatagcaaaattccgcagattatcctgaacatgtgtgaaatctctaaaacctacaacccgtcacgctcggatgacattctgctgctgaaagaactgtattccctgctgtacgcactgatcgaagaatttccgaaaccgtttgaatacaaagataaagaactgcatacctacattcaggacgcgctgaacttcatcaactcaaattatatgcactcgattacggtgcaagaaatcgccgattacgttaatctgagccgttcttacctgtacaaaatgttcatcaaaaacctgggtatcagtccgcagcgttatctgattaatctgcgcatgtacaaagcaaccctgctgctgaaatctacgaaactgccgatcggcgaagttgcgagcagcgtgggttatagtgattccctgctgtttagtaaaaccttctccaaacacttttcaatgtcgccgctgaactaccgcaacaatcaagttaataaaccgagcattggtggtaccggaggcggcttcgaacttcagatggcttccaaggtgtacgaccccgagcaacgcaaacgcatgatcactgggcctcagtggtgggctcgctgcaagcaaatgaacgtgctggactccttcatcaactactatgattccgagaagcacgccgagaacgccgtgatttttctgcatggtaacgctacctccagctacctgtggaggcacgtcgtgcctcacatcgagcccgtggctagatgcatcatccctgatctgatcggaatgggtaagtccggcaagagcgggaatggctcatatcgcctcctggatcactacaagtacctcaccgcttggttcgagctgctgaaccttccaaagaaaatcatctttgtgggccacgactggggggctgctctggcctttcactacgcctacgagcaccaagacaggatcaaggccatcgtccatatggagagtgtcgtggacgtgatcgagtcctgggacgagtggcctgacatcgaggaggatatcgccctgatcaagagcgaagagggcgagaaaatggtgcttgagaataacttcttcgtcgagaccgtgctcccaagcaagatcatgcggaaactggagcctgaggagttcgctgcctacctggagccattcaaggagaagggcgaggttagacggcctaccctctcctggcctcgcgagatccctctcgttaagggaggcaagcccgacgtcgtccagattgtccgcaactacaacgcctaccttcgggccagcgacgatctgcctaagctgttcatcgagtccgaccctgggttcttttccaacgctattgtcgagggagctaagaagttccctaacaccgagttcgtgaaggtgaagggcctccacttcctccaggaggacgctccagatgaaatgggtaagtacatcaagagcttcgtggagcgcgtgctgaagaacgagcagtaa

SEQ ID NO: 31 - DNA, 2640 bp, Artificial Sequence
  Nucleotide sequence encoding LacB3
atgcggggttctcatcatcatcatcatcatggtatggctagcatgactggtggacagcaaatgggtcgggatctgtacgacgatgacgataaggatcgatggggatccgaattcatggtgagcaagggcgaggagctgttcaccggggtggtgcccatcctggtcgagctggacggcgacgtaaacggccacaagttcagcgtgtccggcgagggcgagggcgatgccacctacggcaagctgaccctgaagttcatctgcaccaccggcaagctgcccgtgccctggcccaccctcgtgaccaccctgagctacggcgtgcagtgcttcagccgctaccccgaccacatgaagcagcacgacttcttcaagtccgccatgcccgaaggctacgtccaggagcgcaccatcttcttcaaggacgacggcaactacaagacccgcgccgaggtgaagttcgagggcgacaccctggtgaaccgcatcgagctgaagggcatcgacttcaaggaggacggcaacatcctggggcacaagctggagtacaactacaacagccacaacgtctatatcatggccgacaagcagaagaacggcatcaaggtgaacttcaagatccgccacaacatcgaggacggcagcgtgcagctcgccgaccactaccagcagaacacccccatcggcgacggccccgtgctgctgcccgacaaccactacctgagcacccagtccgccctgagcaaagaccccaacgagaagcgcgatcacatggtcctgctggagttcgtgaccgccgccgggatcactctcggcatggacgagctgtacaagctgcagggtggtaccggaggcggcatgcagattctgtggaaaaaatacgtcaaagaaaactttgaaatgaacgtggatgaatgcggcattgaacaaggcattccgggcctgggttataactacgaagttctgaaaaatgcagtcatccattatgtgaccaaaggctatggtacgtttaaattcaacggcaaagtctataatctgaaacagggtgacattttcatcctgctgaaaggcatgcaagtggaatacgttgcgagcattgatgacccgtgggaatattactggatcggctttagtggttccaacgcgaatgaatatctgaaccgtaccagcattaccaacagctgcgtggccaactgtgaagaaaatagcaaaattccgcagattatcctgaacatgtgtgaaatctctaaaacctacaacccgtcacgctcggatgacattctgctgctgaaagaactgtattccctgctgtacgcactgatcgaagaatttccgaaaccgtttgaatacaaagataaagaactgcatacctacattcaggacgcgctgaacttcatcaactcaaattatatgcactcgattacggtgcaagaaatcgccgattacgttaatctgagccgttcttacctgtacaaaatgttcatcaaaaacctgggtatcagtccgcagcgttatctgattaatctgcgcatgtacaaagcaaccctgctgctgaaatctacgaaactgccgatcggcgaagttgcgagcagcgtgggttatagtgattccctgctgtttagtaaaaccttctccaaacacttttcaatgtcgccgctgaactaccgcaacaatcaagttaataaaccgagcattttcgaacttcagatggcttccaaggtgtacgaccccgagcaacgcaaacgcatgatcactgggcctcagtggtgggctcgctgcaagcaaatgaacgtgctggactccttcatcaactactatgattccgagaagcacgccgagaacgccgtgatttttctgcatggtaacgctacctccagctacctgtggaggcacgtcgtgcctcacatcgagcccgtggctagatgcatcatccctgatctgatcggaatgggtaagtccggcaagagcgggaatggctcatatcgcctcctggatcactacaagtacctcaccgcttggttcgagctgctgaaccttccaaagaaaatcatctttgtgggccacgactggggggctgctctggcctttcactacgcctacgagcaccaagacaggatcaaggccatcgtccatatggagagtgtcgtggacgtgatcgagtcctgggacgagtggcctgacatcgaggaggatatcgccctgatcaagagcgaagagggcgagaaaatggtgcttgagaataacttcttcgtcgagaccgtgctcccaagcaagatcatgcggaaactggagcctgaggagttcgctgcctacctggagccattcaaggagaagggcgaggttagacggcctaccctctcctggcctcgcgagatccctctcgttaagggaggcaagcccgacgtcgtccagattgtccgcaactacaacgcctaccttcgggccagcgacgatctgcctaagctgttcatcgagtccgaccctgggttcttttccaacgctattgtcgagggagctaagaagttccctaacaccgagttcgtgaaggtgaagggcctccacttcctccaggaggacgctccagatgaaatgggtaagtacatcaagagcttcgtggagcgcgtgctgaagaacgagcagtaa

SEQ ID NO: 32 - DNA, 2640 bp, Artificial Sequence
  Nucleotide sequence encoding LacB4
atgcggggttctcatcatcatcatcatcatggtatggctagcatgactggtggacagcaaatgggtcgggatctgtacgacgatgacgataaggatcgatggggatccgaattcatggtgagcaagggcgaggagctgttcaccggggtggtgcccatcctggtcgagctggacggcgacgtaaacggccacaagttcagcgtgtccggcgagggcgagggcgatgccacctacggcaagctgaccctgaagttcatctgcaccaccggcaagctgcccgtgccctggcccaccctcgtgaccaccctgagctacggcgtgcagtgcttcagccgctaccccgaccacatgaagcagcacgacttcttcaagtccgccatgcccgaaggctacgtccaggagcgcaccatcttcttcaaggacgacggcaactacaagacccgcgccgaggtgaagttcgagggcgacaccctggtgaaccgcatcgagctgaagggcatcgacttcaaggaggacggcaacatcctggggcacaagctggagtacaactacaacagccacaacgtctatatcatggccgacaagcagaagaacggcatcaaggtgaacttcaagatccgccacaacatcgaggacggcagcgtgcagctcgccgaccactaccagcagaacacccccatcggcgacggccccgtgctgctgcccgacaaccactacctgagcacccagtccgccctgagcaaagaccccaacgagaagcgcgatcacatggtcctgctggagttcgtgaccgccgccgggatcactctcggcatggacgagctgtacaagctgcagatgcagattctgtggaaaaaatacgtcaaagaaaactttgaaatgaacgtggatgaatgcggcattgaacaaggcattccgggcctgggttataactacgaagttctgaaaaatgcagtcatccattatgtgaccaaaggctatggtacgtttaaattcaacggcaaagtctataatctgaaacagggtgacattttcatcctgctgaaaggcatgcaagtggaatacgttgcgagcattgatgacccgtgggaatattactggatcggctttagtggttccaacgcgaatgaatatctgaaccgtaccagcattaccaacagctgcgtggccaactgtgaagaaaatagcaaaattccgcagattatcctgaacatgtgtgaaatctctaaaacctacaacccgtcacgctcggatgacattctgctgctgaaagaactgtattccctgctgtacgcactgatcgaagaatttccgaaaccgtttgaatacaaagataaagaactgcatacctacattcaggacgcgctgaacttcatcaactcaaattatatgcactcgattacggtgcaagaaatcgccgattacgttaatctgagccgttcttacctgtacaaaatgttcatcaaaaacctgggtatcagtccgcagcgttatctgattaatctgcgcatgtacaaagcaaccctgctgctgaaatctacgaaactgccgatcggcgaagttgcgagcagcgtgggttatagtgattccctgctgtttagtaaaaccttctccaaacacttttcaatgtcgccgctgaactaccgcaacaatcaagttaataaaccgagcattggtggtaccggaggcggcttcgaacttcagatggcttccaaggtgtacgaccccgagcaacgcaaacgcatgatcactgggcctcagtggtgggctcgctgcaagcaaatgaacgtgctggactccttcatcaactactatgattccgagaagcacgccgagaacgccgtgatttttctgcatggtaacgctacctccagctacctgtggaggcacgtcgtgcctcacatcgagcccgtggctagatgcatcatccctgatctgatcggaatgggtaagtccggcaagagcgggaatggctcatatcgcctcctggatcactacaagtacctcaccgcttggttcgagctgctgaaccttccaaagaaaatcatctttgtgggccacgactggggggctgctctggcctttcactacgcctacgagcaccaagacaggatcaaggccatcgtccatatggagagtgtcgtggacgtgatcgagtcctgggacgagtggcctgacatcgaggaggatatcgccctgatcaagagcgaagagggcgagaaaatggtgcttgagaataacttcttcgtcgagaccgtgctcccaagcaagatcatgcggaaactggagcctgaggagttcgctgcctacctggagccattcaaggagaagggcgaggttagacggcctaccctctcctggcctcgcgagatccctctcgttaagggaggcaagcccgacgtcgtccagattgtccgcaactacaacgcctaccttcgggccagcgacgatctgcctaagctgttcatcgagtccgaccctgggttcttttccaacgctattgtcgagggagctaagaagttccctaacaccgagttcgtgaaggtgaagggcctccacttcctccaggaggacgctccagatgaaatgggtaagtacatcaagagcttcgtggagcgcgtgctgaagaacgagcagtaa

SEQ ID NO: 33 - protein, 765 aa, Artificial Sequence
  GFP2-BgaR1-171-RLuc8
MRGSHHHHHHGMASMTGGQQMGRDLYDDDDKDRWGSEFMVSKGEELFTGVVPILVELDGDVNGHKFSVSGEGEGDATYGKLTLKFICTTGKLPVPWPTLVTTLSYGVQCFSRYPDHMKQHDFFKSAMPEGYVQERTIFFKDDGNYKTRAEVKFEGDTLVNRIELKGIDFKEDGNILGHKLEYNYNSHNVYIMADKQKNGIKVNFKIRHNIEDGSVQLADHYQQNTPIGDGPVLLPDNHYLSTQSALSKDPNEKRDHMVLLEFVTAAGITLGMDELYKLQMQILWKKYVKENFEMNVDECGIEQGIPGLGYNYEVLKNAVIHYVTKGYGTFKFNGKVYNLKQGDIFILLKGMQVEYVASIDDPWEYYWIGFSGSNANEYLNRTSITNSCVANCEENSKIPQIILNMCEISKTYNPSRSDDILLLKELYSLLYALIEEFPKPFEYKDKELHTFELQMASKVYDPEQRKRMITGPQWWARCKQMNVLDSFINYYDSEKHAENAVIFLHGNATSSYLWRHVVPHIEPVARCIIPDLIGMGKSGKSGNGSYRLLDHYKYLTAWFELLNLPKKIIFVGHDWGAALAFHYAYEHQDRIKAIVHMESVVDVIESWDEWPDIEEDIALIKSEEGEKMVLENNFFVETVLPSKIMRKLEPEEFAAYLEPFKEKGEVRRPTLSWPREIPLVKGGKPDVVQIVRNYNAYLRASDDLPKLFIESDPGFFSNAIVEGAKKFPNTEFVKVKGLHFLQEDAPDEMGKYIKSFVERVLKNEQ

SEQ ID NO: 34 - protein, 744 aa, Artificial Sequence
  GFP2-BgaR1-150-RLuc8
MRGSHHHHHHGMASMTGGQQMGRDLYDDDDKDRWGSEFMVSKGEELFTGVVPILVELDGDVNGHKFSVSGEGEGDATYGKLTLKFICTTGKLPVPWPTLVTTLSYGVQCFSRYPDHMKQHDFFKSAMPEGYVQERTIFFKDDGNYKTRAEVKFEGDTLVNRIELKGIDFKEDGNILGHKLEYNYNSHNVYIMADKQKNGIKVNFKIRHNIEDGSVQLADHYQQNTPIGDGPVLLPDNHYLSTQSALSKDPNEKRDHMVLLEFVTAAGITLGMDELYKLQMQILWKKYVKENFEMNVDECGIEQGIPGLGYNYEVLKNAVIHYVTKGYGTFKFNGKVYNLKQGDIFILLKGMQVEYVASIDDPWEYYWIGFSGSNANEYLNRTSITNSCVANCEENSKIPQIILNMCEISKTYNPSRSDDILLLKELYSLFELQMASKVYDPEQRKRMITGPQWWARCKQMNVLDSFINYYDSEKHAENAVIFLHGNATSSYLWRHVVPHIEPVARCIIPDLIGMGKSGKSGNGSYRLLDHYKYLTAWFELLNLPKKIIFVGHDWGAALAFHYAYEHQDRIKAIVHMESVVDVIESWDEWPDIEEDIALIKSEEGEKMVLENNFFVETVLPSKIMRKLEPEEFAAYLEPFKEKGEVRRPTLSWPREIPLVKGGKPDVVQIVRNYNAYLRASDDLPKLFIESDPGFFSNAIVEGAKKFPNTEFVKVKGLHFLQEDAPDEMGKYIKSFVERVLKNEQ

SEQ ID NO: 35 - protein, 754 aa, Artificial Sequence
  GFP2-BgaR12-171-RLuc8
MRGSHHHHHHGMASMTGGQQMGRDLYDDDDKDRWGSEFMVSKGEELFTGVVPILVELDGDVNGHKFSVSGEGEGDATYGKLTLKFICTTGKLPVPWPTLVTTLSYGVQCFSRYPDHMKQHDFFKSAMPEGYVQERTIFFKDDGNYKTRAEVKFEGDTLVNRIELKGIDFKEDGNILGHKLEYNYNSHNVYIMADKQKNGIKVNFKIRHNIEDGSVQLADHYQQNTPIGDGPVLLPDNHYLSTQSALSKDPNEKRDHMVLLEFVTAAGITLGMDELYKLQNFEMNVDECGIEQGIPGLGYNYEVLKNAVIHYVTKGYGTFKFNGKVYNLKQGDIFILLKGMQVEYVASIDDPWEYYWIGFSGSNANEYLNRTSITNSCVANCEENSKIPQIILNMCEISKTYNPSRSDDILLLKELYSLLYALIEEFPKPFEYKDKELHTFELQMASKVYDPEQRKRMITGPQWWARCKQMNVLDSFINYYDSEKHAENAVIFLHGNATSSYLWRHVVPHIEPVARCIIPDLIGMGKSGKSGNGSYRLLDHYKYLTAWFELLNLPKKIIFVGHDWGAALAFHYAYEHQDRIKAIVHMESVVDVIESWDEWPDIEEDIALIKSEEGEKMVLENNFFVETVLPSKIMRKLEPEEFAAYLEPFKEKGEVRRPTLSWPREIPLVKGGKPDVVQIVRNYNAYLRASDDLPKLFIESDPGFFSNAIVEGAKKFPNTEFVKVKGLHFLQEDAPDEMGKYIKSFVERVLKNEQ

SEQ ID NO: 36 - protein, 733 aa, Artificial Sequence
  GFP2-BgaR12-150-RLuc8
MRGSHHHHHHGMASMTGGQQMGRDLYDDDDKDRWGSEFMVSKGEELFTGVVPILVELDGDVNGHKFSVSGEGEGDATYGKLTLKFICTTGKLPVPWPTLVTTLSYGVQCFSRYPDHMKQHDFFKSAMPEGYVQERTIFFKDDGNYKTRAEVKFEGDTLVNRIELKGIDFKEDGNILGHKLEYNYNSHNVYIMADKQKNGIKVNFKIRHNIEDGSVQLADHYQQNTPIGDGPVLLPDNHYLSTQSALSKDPNEKRDHMVLLEFVTAAGITLGMDELYKLQNFEMNVDECGIEQGIPGLGYNYEVLKNAVIHYVTKGYGTFKFNGKVYNLKQGDIFILLKGMQVEYVASIDDPWEYYWIGFSGSNANEYLNRTSITNSCVANCEENSKIPQIILNMCEISKTYNPSRSDDILLLKELYSLFELQMASKVYDPEQRKRMITGPQWWARCKQMNVLDSFINYYDSEKHAENAVIFLHGNATSSYLWRHVVPHIEPVARCIIPDLIGMGKSGKSGNGSYRLLDHYKYLTAWFELLNLPKKIIFVGHDWGAALAFHYAYEHQDRIKAIVHMESVVDVIESWDEWPDIEEDIALIKSEEGEKMVLENNFFVETVLPSKIMRKLEPEEFAAYLEPFKEKGEVRRPTLSWPREIPLVKGGKPDVVQIVRNYNAYLRASDDLPKLFIESDPGFFSNAIVEGAKKFPNTEFVKVKGLHFLQEDAPDEMGKYIKSFVERVLKNEQ

SEQ ID NO: 37 - protein, 279 aa, Artificial Sequence
  A0A133MUX6
MQILWKKYVKENFEMNVDECGIEQGIPGLGYNYEVLKNAVIHYVTKGYGTFKFNGKVYNLKQGDIFILLKGMQVEYVASIDDPWEYYWIGFSGSNANEYLNRTSITDSCVANCEENSKIPQIILNMCEISKTYNPSRSDDILLLKELYSLLYALIEEFPKPFEYKDKELHTYIQDALNFINSNYMHSITVQEIADYVNLSRSYLYKMFIKNLGISPQRYLINLRMYKATLLLKGTKLPIGEVASSVGYSDSLLFSKTFSKHFSMSPLNYRNNQVNKPNI

SEQ ID NO: 38 - protein, 279 aa, Artificial Sequence
  B1V7N0
MQILWKKYVKENFEMNVDECGIEQGIPGLGYKYEVLKNAVIHYVTKGYGTFKFNGKVYTLKQGDIFILLKGMQVDYVASIDDPWEYYWIGFSGSNANEYLNRTSITNSCVANCEENSKIPQIILNMCEISKTYNPSRSDDILLLKELYSLLYALIEEFPKPFEYKDKELHTYIQDALNFINSNYMHSITVQEIADYVNLSRSYLYKMFIKNLGISPQRYLINLRMYKATLLLKGTKLPIGEVASSVGYSDSLLFSKTFSKHFSMSPLNYRNNQVYKSSI

SEQ ID NO: 39 - protein, 279 aa, Artificial Sequence
  A0A127EGD8
MQILWKKYIKENFEMNVDECGIEQGIPGLGYKYEVLKNAVIHYVTKGYGTFKFNGKVYTLKQGDIFILLKGMKVEYVASIDDPWEYYWIGFSGSNANEYLNRTSITNSYVANCEKNSKIPQIILNMCEISKTYNPSSSDDILLLKELYSLLYTLIEEFPKPFDYKDKELHTYIQDALNFINSNYMNSITVQEIADYVNLSRSYLYKMFIKNLGISPQRYLINLRMYKATLLLKGTKLPIGEVASRIGYSDSLLFSKTFSKHFSMSPLNYRNNQVNKPSI

SEQ ID NO: 40 - protein, 278 aa, Artificial Sequence
  A0A1C6JUB7
MQILWKKYTKENFEMNVDECGIEQGIPGFGYKYEVLKNAVIHYISKGNGTFKFNDKVYNLKQGDVFILLKGMKVEYIASIDDPWEYYWIGFSGSNANEYLNRTSIIDSYAANCKEDSKIPDIISNMCEISKTYNPSRSDDILLLKELYSLLYAFIEEFPKAFEYKDKELHTYIQEAIDFINSNYMNSITVNDIAEHVNLSRSYLYKMFMKNLKVSPQKYLINLRMYKATLLLKNTRIPIGEVASKVGYSDSLLFSKTFSKYFSMSPLNYRNNQMNGNK

SEQ ID NO: 41 - protein, 278 aa, Artificial Sequence
  A0A174HYB7
MQILWKKYTKENFEMNVDECGIEQGIPGFGYKYEVLKNAVIHYISKGNGTFKFNDKVYNLKQGDVFILLKGMKVEYIASIDDPWEYYWIGFSGSNANEYLNRTSIIDSYAAKCKGDSKIPDIISNMCEISKTYNPSRSDDILLLKELYSLLYAFIEEFPKAFEYKDKELHTYIQEAIDFINSNYMNSITVNDIAEHINLSRSYLYKMFMKNLKVSPQKYLINLRMYKATLLLKGTRIPIGEVASKVGYSDSLLFSKTFSKYFSMSPLNYRNNQTSDNK

SEQ ID NO: 42 - protein, 278 aa, Artificial Sequence
  A0A1C6KY47
MQILWKKYIKENFEMNVDECGIEQGIPGFGYKYEVLKNSVIHYITKGHGTFKINDKLYNLGQGDVFILLKGMKVEYMASIDDPWEYYWIGFSGSNANEYLNRTSIIDSYAATCKEDSKIPCIISNMCEISKTYNPSCCDDILLLKELYSLLYAFIEEFPKAFEYKDKELHTYIQEAINFINSNYMKSITVNDIAEHVNLSRSYLYKMFMKNLKVSPQKYLINLRMYKATLLLKGTRIPIGEVASKVGYSDSLLFSKTFSKYFSMSPLNYRNNQTSDNK

SEQ ID NO: 43 - protein, 277 aa, Artificial Sequence
  A0A174LZQ7
MQILWRKYKKENFDINLDECGIEHGIPGFGYRYKVLKNSVIHYVIRGYGTFKVNDKVYNLKEGDIFILLKGMDVEYMASMDNPWEYCWIGFSGSKADEYLNRTSIIDSHVANCNENSKIPCIILNICEISKNYNPSNSDDILLLNELYSLLYELIGEFPKPFEYKDKEIHKYIQDTINFINSNYMNNITVNEIAEHVNLSRSYLYKMFIKNLKISPQKYLINLRMYKATLLLKNTKLPIGEIANKVGYADSLLFSKTFSKYFSVSPLNYRNNKVNKE

SEQ ID NO: 44 - protein, 279 aa, Artificial Sequence
  N9YR91
MQILWKKYKNINFDSNLDECGIEQGTPGTGYKYEVVKNAVIHYISKGSGIFKINDKIYNLKRGDGFILLKGMHVEYISSIDDPWKYYWVGFSGKNANEYLKRTSIIDTCIINFSKKSKVPNTIIDMCNISKKYNQTSSDDILLLSKLHLLLYYISSEFPKSFKYYNNLAHTYIQEAVDFINNNYMKSITVQEVANHVNLSRSYLYKMFIKYLGQSTQSYLINIRMYKSSLLLKETNLSILEIANKVGYDDPGLFSKTFSKHFSMSASKYRKIYQKNKTN

SEQ ID NO: 45 - protein, 279 aa, Artificial Sequence
  A0A174I591
MQILWNKYKSNNFEANLDECGIEQGTPGAGYNYKVEKNAVIHYISKGSGTFKINDKIYTLKKGDGFILLKDMNVEYIPSIDDPWKYYWIGFSGQSLNEYLKRTSIIDSCVINFSKKSKIPNLIIDMCNISKKYDQTSSDDILLLSKLHLLLYYISSEFPKAFKYNNNLTHTYIQEATTFINNNYMNPITVQEVADHVNLSRSYLYKMFIKHLGESTQSYLINIRMYKSSILLKETSLSIAEIANKVGYSDPLLFSKIFSKHFSMSASKYRKSHQKNKKC

SEQ ID NO: 46 - protein, 275 aa, Artificial Sequence
  A0A2A7ME67
MQILWKKYKITNFEMNLDECGIEQCTPGIKYNYEVVKNSVIHYISEGEGTFKINNQIFDLKKGDGFILFKGMNVEYTASIDNPWKYYWVGFSGTNANEYLHRSSIFDNYIINYQSNSKIPSIIKNMCALSKTYDQNSSDDILLLNKLYYLLYTITQEFPKPFQLVNNLTHTYIQQSIDFINSKYAEKITVQQIADNVNLSRSYLYKLFIKYLGESPQKYLLNLRMYKATLLLKETDLSISQISSNIGYDDPLFFSKTFSKHFSISASQYRKLYKK

SEQ ID NO: 47 - protein, 274 aa, Artificial Sequence
  A0A2K4AZL9
MQLLWKMFKKNQFEANIDECGIEIGTPQGGYQYEVTKPAVLHVVMSGTGTLTYNQKKYTLKPGDLFLLCRGMKVHYESTLDEPWTYYWVGFSGKLAMDYLNRTTLYETRVIQNQQTSTIRQIIYQMCHRSIDYNPEHSDDIQHMRDLYDLLYALHQHFPKPFHVVKNEKYSNVREAIRYINDNYMHGISIHDVAKHVNVSRSYLYKMFKKHIDQSPQHYLIHIRMYHASQLFKDTDLQSQEIADRVGYKDPLLFSRAFKKHFGITATQYRETHQ

SEQ ID NO: 48 - protein, 286 aa, Artificial Sequence
  A0A166PPM9
MQLLWKMFKKNQFEANIDECGIEIGTPHGGYQYEVTKPAVLHIVMSGTGTLTYNQKKYTLKPGDLFLLCRGMNVHYESTLDEPWTYYWVGFSGKLVFDYLNRTSLYETRVIQNQPTNTIRQIIYRMCQRSIEYATENSDDIQHMRDLYELLYELHQHFPKPFHVVKNERYSNVREAIRYINDNYMHAISINDVAKHVNVSRSYLYKMFKKHIDQSPQHYLIHIRMYHASQLFKETDLQSQEIADRVGYKDPLLFSRAFKKHFGVTATQYREEQQLRIESTLDNQKR

SEQ ID NO: 49 - protein, 274 aa, Artificial Sequence
  A0A2T4R7G1
MQLLWKLFKRNHFEANIDECGIEIGTPNVSYQYTVVKPAVLHIIVAGTGSFTYQQSTYQLKSGDMFLLQEGMHVHYEASADDPWTYHWVGFSGNLAIDYLKRTSLIDCPVVMNKDTSDISKVMYQICERAITYETATSDDIHHLSDLYKLLFLITQCAPKPFEKEHNEIYSSVQDAVDYMNQNYMYAITIDDIAQYAKVSRSYLYKLFIKWMDQSPQQYLIYLRLYHASSMLKTTSKPIQDIAQAVGYSDPLLFSKAFRKHFDMPPSTYRKVYK

SEQ ID NO: 50 - protein, 274 aa, Artificial Sequence
  A0A2A4HCU9
MQLLWKMFKKNQFEANIDECGIEIGTPQRGYQYEVTKPAVLHVVMSGTGTLTYNQKKYTLKPGDLFLLCRGMNVHYESTLDEPWTYYWVGFSGKLVFDYLNRTSLYETRVIQNQPTNAIRQIIYRMCHRSIEYATENSDDIQHMRDLYELLYELHQHFPKPFHVVKNEKYSNVREAIRYMNDNYMHAISINDVAKHVNVSRSYLYKMFKKHIDQSPQHYLIHIRMYHASQLFKETDLQSQEIADRVGYKDPLLFSRAFKKHFGVTATQYREEHQ

SEQ ID NO: 51 - protein, 271 aa, Artificial Sequence
  A0A2T4MS83
MQLLWKLFKKNHFEANIDECGIEIGTPNVSYQYTVVKPAVLHIIMSGTGTFTHQHTSYELKAGDMFLLREGMRVHYEASTDDPWTYHWVGFSGNLAMDYLKRTTLIDCPVVLNQDTSKLSKLMYQICERAITYETTASDDIHHLSDLYKLLFLLTQLSPKPFESHPNEIYSSVQAAVNYMNQHYMHTISIDDVAQHAKVSRSYLYKLFMKWMDQSPQQYLVYLRLYHASSMLKTTSKPIQEIAQNVGYNDPLLFSKAFRKHFDMPPSTYRK

SEQ ID NO: 52 - protein, 279 aa, Artificial Sequence
  O33813
MQVLWKKFQKKLIDANLAECGIEIGVPNVGYNYTVFQKSVLHIVTQGEGTFSYAGETYHLTAGDIFLLERGMEVEYKPSFSNPWTYYWVGMNGKQILNYLSRCSIVDSHVILGQDTTDIKNIIQLICKLSQSIESNNSNDILIMQYLYQLVYTLQEKFPKIFSVQVDIVNEDIQHAVDFINTNYQKHITVEDVAKSVNITRSHLYKLFKKNLGCSPKEYLTYIRMYHASQLLIHTSTLISDISRQVGYKDPLLFSKNFTKHFEISASEYRHHFSINNKQ

SEQ ID NO: 53 - protein, 277 aa, Artificial Sequence
  A0A1D4LKB2
MQILWKKFQKKLVDANLAECGIEIGIPNVGYDYTVLQQSVLHIVTDGEGVFKYNNEIYHLKKGDIFLLERGMSVKYMPSFSNPWTYYWVGINGKQLLNYLMRSYIVDTHVIIGKDTQDIKVIIQKLCKLAKDIQSTNSNDILIMQYLYKLVYTFQDKFPKTFTVPLDIVNEDIQHAIEFINTHYQNGITITDVTNSVNMSRSYLYKLFKKHLNCSPKSYLTYIRMYHASQLLINSNLLVSEISQRVGYSDPLLFSKNFTKHFEISASAYRFHFQQNK

SEQ ID NO: 54 - protein, 314 aa, Artificial Sequence
  A0A133QVV5
MTLLSIFQKLYNFVKYTCYNGSIIERKRVRQVQVFWTKLKKTSYEAQVDECGKENLYVGNGYEYEVTKPAVLHIVTQGTGTFTVNDTTYHLKKGDVFLLLKGMHVKYHATGETPWHYMWVGFSGTHAISFITRTSLSDEFVLLNQNTETLFKLIFKICILANSHTPEDTHDILLKIRLFELLYFLTQQNQKEIVIPDQREATDLKDALEYFNDNFKSKDTTVDNAAQVANMSRSQLYKRFKKQFGASPSRYLTDLRMAFAAEQLKFTNKTVQAIADELNYDVSLAFSKAFSKYFNCPPTQYRKNYKARKALQSE

SEQ ID NO: 55 - protein, 289 aa, Artificial Sequence
  A9QSR3
MEYKEFHQNFLDINLDFVGNEATIPNFSFGPAIRENYVIHYITSGSGRYMIYGFEHQLKAGDCFIIPADVETFYQSDALTPWAYYWLGLSGHVVNDLFARTALDDKGWILENVSKTEFIEHFSKIQNLISDDDKTVDLDIQVELFALMKSLITLFPKSITEHKNQSDYYAEKAYTFINQNYSQSIKIKDVLAHVMISRAYLFTIFKHKYGLSPQKYLIDLRMAKAAMLLIHSDNLVSQISEAVGFSDSLSFSSAFKKRYGVSPTKFKTQKHDNLMLETLNNMNLNRLKK

SEQ ID NO: 56 - protein, 139 aa, Artificial Sequence
  A0A133MUX6 CBD
NFEMNVDECGIEQGIPGLGYNYEVLKNAVIHYVTKGYGTFKFNGKVYNLKQGDIFILLKGMQVEYVASIDDPWEYYWIGFSGSNANEYLNRTSITDSCVANCEENSKIPQIILNMCEISKTYNPSRSDDILLLKELYSL

SEQ ID NO: 57 - protein, 139 aa, Artificial Sequence
  B1V7N0 CBD
NFEMNVDECGIEQGIPGLGYKYEVLKNAVIHYVTKGYGTFKFNGKVYTLKQGDIFILLKGMQVDYVASIDDPWEYYWIGFSGSNANEYLNRTSITNSCVANCEENSKIPQIILNMCEISKTYNPSRSDDILLLKELYSL

SEQ ID NO: 58 - protein, 139 aa, Artificial Sequence
  A0A127EGD8 CBD
NFEMNVDECGIEQGIPGLGYKYEVLKNAVIHYVTKGYGTFKFNGKVYTLKQGDIFILLKGMKVEYVASIDDPWEYYWIGFSGSNANEYLNRTSITNSYVANCEKNSKIPQIILNMCEISKTYNPSSSDDILLLKELYSL

SEQ ID NO: 59 - protein, 139 aa, Artificial Sequence
  A0A1C6JUB7 CBD
NFEMNVDECGIEQGIPGFGYKYEVLKNAVIHYISKGNGTFKFNDKVYNLKQGDVFILLKGMKVEYIASIDDPWEYYWIGFSGSNANEYLNRTSIIDSYAANCKEDSKIPDIISNMCEISKTYNPSRSDDILLLKELYSL

SEQ ID NO: 60 - protein, 139 aa, Artificial Sequence
  A0A174HYB7 CBD
NFEMNVDECGIEQGIPGFGYKYEVLKNAVIHYISKGNGTFKFNDKVYNLKQGDVFILLKGMKVEYIASIDDPWEYYWIGFSGSNANEYLNRTSIIDSYAAKCKGDSKIPDIISNMCEISKTYNPSRSDDILLLKELYSL

SEQ ID NO: 61 - protein, 139 aa, Artificial Sequence
  A0A1C6KY47 CBD
NFEMNVDECGIEQGIPGFGYKYEVLKNSVIHYITKGHGTFKINDKLYNLGQGDVFILLKGMKVEYMASIDDPWEYYWIGFSGSNANEYLNRTSIIDSYAATCKEDSKIPCIISNMCEISKTYNPSCCDDILLLKELYSL

SEQ ID NO: 62 - protein, 139 aa, Artificial Sequence
  A0A174LZQ7 CBD
NFDINLDECGIEHGIPGFGYRYKVLKNSVIHYVIRGYGTFKVNDKVYNLKEGDIFILLKGMDVEYMASMDNPWEYCWIGFSGSKADEYLNRTSIIDSHVANCNENSKIPCIILNICEISKNYNPSNSDDILLLNELYSL

SEQ ID NO: 63 - protein, 139 aa, Artificial Sequence
  N9YR91 CBD
NFDSNLDECGIEQGTPGTGYKYEVVKNAVIHYISKGSGIFKINDKIYNLKRGDGFILLKGMHVEYISSIDDPWKYYWVGFSGKNANEYLKRTSIIDTCIINFSKKSKVPNTIIDMCNISKKYNQTSSDDILLLSKLHLL

SEQ ID NO: 64 - protein, 139 aa, Artificial Sequence
  A0A174I591 CBD
NFEANLDECGIEQGTPGAGYNYKVEKNAVIHYISKGSGTFKINDKIYTLKKGDGFILLKDMNVEYIPSIDDPWKYYWIGFSGQSLNEYLKRTSIIDSCVINFSKKSKIPNLIIDMCNISKKYDQTSSDDILLLSKLHLL

SEQ ID NO: 65 - protein, 139 aa, Artificial Sequence
  A0A2A7ME67 CBD
NFEMNLDECGIEQCTPGIKYNYEVVKNSVIHYISEGEGTFKINNQIFDLKKGDGFILFKGMNVEYTASIDNPWKYYWVGFSGTNANEYLHRSSIFDNYIINYQSNSKIPSIIKNMCALSKTYDQNSSDDILLLNKLYYL

SEQ ID NO: 66 - protein, 139 aa, Artificial Sequence
  A0A2K4AZL9 CBD
QFEANIDECGIEIGTPQGGYQYEVTKPAVLHVVMSGTGTLTYNQKKYTLKPGDLFLLCRGMKVHYESTLDEPWTYYWVGFSGKLAMDYLNRTTLYETRVIQNQQTSTIRQIIYQMCHRSIDYNPEHSDDIQHMRDLYDL

SEQ ID NO: 67 - protein, 139 aa, Artificial Sequence
  A0A166PPM9 CBD
QFEANIDECGIEIGTPHGGYQYEVTKPAVLHIVMSGTGTLTYNQKKYTLKPGDLFLLCRGMNVHYESTLDEPWTYYWVGFSGKLVFDYLNRTSLYETRVIQNQPTNTIRQIIYRMCQRSIEYATENSDDIQHMRDLYEL

SEQ ID NO: 68 - protein, 139 aa, Artificial Sequence
  A0A2T4R7G1 CBD
HFEANIDECGIEIGTPNVSYQYTVVKPAVLHIIVAGTGSFTYQQSTYQLKSGDMFLLQEGMHVHYEASADDPWTYHWVGFSGNLAIDYLKRTSLIDCPVVMNKDTSDISKVMYQICERAITYETATSDDIHHLSDLYKL

SEQ ID NO: 69 - protein, 139 aa, Artificial Sequence
  A0A2A4HCU9 CBD
QFEANIDECGIEIGTPQRGYQYEVTKPAVLHVVMSGTGTLTYNQKKYTLKPGDLFLLCRGMNVHYESTLDEPWTYYWVGFSGKLVFDYLNRTSLYETRVIQNQPTNAIRQIIYRMCHRSIEYATENSDDIQHMRDLYEL

SEQ ID NO: 70 - protein, 139 aa, Artificial Sequence
  A0A2T4MS83 CBD
HFEANIDECGIEIGTPNVSYQYTVVKPAVLHIIMSGTGTFTHQHTSYELKAGDMFLLREGMRVHYEASTDDPWTYHWVGFSGNLAMDYLKRTTLIDCPVVLNQDTSKLSKLMYQICERAITYETTASDDIHHLSDLYKL

SEQ ID NO: 71 - protein, 139 aa, Artificial Sequence
  O33813 CBD
LIDANLAECGIEIGVPNVGYNYTVFQKSVLHIVTQGEGTFSYAGETYHLTAGDIFLLERGMEVEYKPSFSNPWTYYWVGMNGKQILNYLSRCSIVDSHVILGQDTTDIKNIIQLICKLSQSIESNNSNDILIMQYLYQL

SEQ ID NO: 72 - protein, 139 aa, Artificial Sequence
  A0A1D4LKB2 CBD
LVDANLAECGIEIGIPNVGYDYTVLQQSVLHIVTDGEGVFKYNNEIYHLKKGDIFLLERGMSVKYMPSFSNPWTYYWVGINGKQLLNYLMRSYIVDTHVIIGKDTQDIKVIIQKLCKLAKDIQSTNSNDILIMQYLYKL

SEQ ID NO: 73 - protein, 139 aa, Artificial Sequence
  A0A133QVV5 CBD
NFVKYTCYNGSIIERKRVRQVQVFWTKLKKTSYEAQVDECGKENLYVGNGYEYEVTKPAVLHIVTQGTGTFTVNDTTYHLKKGDVFLLLKGMHVKYHATGETPWHYMWVGFSGTHAISFITRTSLSDEFVLLNQNTETL

SEQ ID NO: 74 - protein, 139 aa, Artificial Sequence
  A9QSR3
DINLDFVGNEATIPNFSFGPAIRENYVIHYITSGSGRYMIYGFEHQLKAGDCFIIPADVETFYQSDALTPWAYYWLGLSGHVVNDLFARTALDDKGWILENVSKTEFIEHFSKIQNLISDDDKTVDLDIQVELFALMKS